European Patent Application EP 4 520 823 A1, published March 12, 2025. Title: UTR sequence for controlling protein expression and protein localization, and mRNA sequence comprising the same. Applicant: Industry-Academic Cooperation Foundation, Dankook University. The sequence listing filed with the application follows.

SEQUENCE LISTING (77 sequences)

SEQ ID NO: 1 - RNA, 268 nt, Homo sapiens
  source 1..268: mol_type = mRNA
aggatacagcggcttctgcgcgacttataagagctccttgtgcggcgccattttaagcctctcggtctgtggcagcagcgttggcccggccccgggagcggagagcgaggggaggcggagacggaggaaggtctgaggagcagcttcagtccccgccgagccgccaccgcaggtcgaggacggtcggactcccgcggcgggaggagcctgttcccctgagggtatttgaagtataccatacaactgttttgaaaatccagcgtggaca

SEQ ID NO: 2 - RNA, 12 nt, Homo sapiens
  source 1..12: mol_type = mRNA
atcatcctttag

SEQ ID NO: 3 - RNA, 305 nt, Homo sapiens
  source 1..305: mol_type = mRNA
gtaagaagttttaaaaagccagtttgggtaaaatacttttactctgcctacagaacttcagaaagacttggttggtagggtgggagtggtttaggctatttgtaaatctgccacaaaaacaggtatatactttgaaaggagatgtcttggaacattggaatgttctcagatttctggttgttatgtgatcatgtgtggaagttattaactttaatgttttttgccacagcttttgcaacttaatactcaaatgagtaacatttgctgttttaaacattaatagcagcctttctctctttatacag

SEQ ID NO: 4 - RNA, 159 nt, Homo sapiens
  source 1..159: mol_type = mRNA
ctgtattgtctgaacttgcattgtgattggcctgtagagttgctgagagggctcgaggggtgggctggtatctcagaaagtgcctgacacactaaccaagctgagtttcctatgggaacaattgaagtaaactttttgttctggtcctttttggtcgag

SEQ ID NO: 5 - RNA, 625 nt, Homo sapiens
  source 1..625: mol_type = mRNA
gagtaacaatacaaatggattttgggagtgactcaagaagtgaagaatgcacaagaatggatcacaagatggaatttatcaaaccctagccttgcttgttaaatttttttttttttttttttaagaatatctgtaatggtactgactttgcttgctttgaagtagctctttttttttttttttttttttttttgcagtaactgttttttaagtctctcgtagtgttaagttatagtgaatactgctacagcaatttctaatttttaagaattgagtaatggtgtagaacactaattcataatcactctaattaattgtaatctgaataaagtgtaacaattgtgtagcctttttgtataaaatagacaaatagaaaatggtccaattagtttcctttttaatatgcttaaaataagcaggtggatctatttcatgtttttgatcaaaaactatttgggatatgtatgggtagggtaaatcagtaagaggtgttatttggaaccttgttttggacagtttaccagttgccttttatcccaaagttgttgtaacctgctgtgatacgatgcttcaagagaaaatgcggttataaaaaatggttcagaattaaacttttaattcattc

SEQ ID NO: 6 - RNA, 642 nt, Homo sapiens
  source 1..642: mol_type = mRNA
atcatcctttaggagtaacaatacaaatggattttgggagtgactcaagaagtgaagaatgcacaagaatggatcacaagatggaatttatcaaaccctagccttgcttgttaaatttttttttttttttttttaagaatatctgtaatggtactgactttgcttgctttgaagtagctctttttttttttttttttttttttttgcagtaactgttttttaagtctctcgtagtgttaagttatagtgaatactgctacagcaatttctaatttttaagaattgagtaatggtgtagaacactaattcataatcactctaattaattgtaatctgaataaagtgtaacaattgtgtagcctttttgtataaaatagacaaatagaaaatggtccaattagtttcctttttaatatgcttaaaataagcaggtggatctatttcatgtttttgatcaaaaactatttgggatatgtatgggtagggtaaatcagtaagaggtgttatttggaaccttgttttggacagtttaccagttgccttttatcccaaagttgttgtaacctgctgtgatacgatgcttcaagagaaaatgcggttataaaaaatggttcagaattaaacttttaattcattcgattg

SEQ ID NO: 7 - RNA, 801 nt, Homo sapiens
  source 1..801: mol_type = mRNA
atcatcctttagctgtattgtctgaacttgcattgtgattggcctgtagagttgctgagagggctcgaggggtgggctggtatctcagaaagtgcctgacacactaaccaagctgagtttcctatgggaacaattgaagtaaactttttgttctggtcctttttggtcgaggagtaacaatacaaatggattttgggagtgactcaagaagtgaagaatgcacaagaatggatcacaagatggaatttatcaaaccctagccttgcttgttaaatttttttttttttttttttaagaatatctgtaatggtactgactttgcttgctttgaagtagctctttttttttttttttttttttttttgcagtaactgttttttaagtctctcgtagtgttaagttatagtgaatactgctacagcaatttctaatttttaagaattgagtaatggtgtagaacactaattcataatcactctaattaattgtaatctgaataaagtgtaacaattgtgtagcctttttgtataaaatagacaaatagaaaatggtccaattagtttcctttttaatatgcttaaaataagcaggtggatctatttcatgtttttgatcaaaaactatttgggatatgtatgggtagggtaaatcagtaagaggtgttatttggaaccttgttttggacagtttaccagttgccttttatcccaaagttgttgtaacctgctgtgatacgatgcttcaagagaaaatgcggttataaaaaatggttcagaattaaacttttaattcattcgattg

SEQ ID NO: 8 - RNA, 1106 nt, Homo sapiens
  source 1..1106: mol_type = mRNA
atcatcctttaggtaagaagttttaaaaagccagtttgggtaaaatacttttactctgcctacagaacttcagaaagacttggttggtagggtgggagtggtttaggctatttgtaaatctgccacaaaaacaggtatatactttgaaaggagatgtcttggaacattggaatgttctcagatttctggttgttatgtgatcatgtgtggaagttattaactttaatgttttttgccacagcttttgcaacttaatactcaaatgagtaacatttgctgttttaaacattaatagcagcctttctctctttatacagctgtattgtctgaacttgcattgtgattggcctgtagagttgctgagagggctcgaggggtgggctggtatctcagaaagtgcctgacacactaaccaagctgagtttcctatgggaacaattgaagtaaactttttgttctggtcctttttggtcgaggagtaacaatacaaatggattttgggagtgactcaagaagtgaagaatgcacaagaatggatcacaagatggaatttatcaaaccctagccttgcttgttaaatttttttttttttttttttaagaatatctgtaatggtactgactttgcttgctttgaagtagctctttttttttttttttttttttttttgcagtaactgttttttaagtctctcgtagtgttaagttatagtgaatactgctacagcaatttctaatttttaagaattgagtaatggtgtagaacactaattcataatcactctaattaattgtaatctgaataaagtgtaacaattgtgtagcctttttgtataaaatagacaaatagaaaatggtccaattagtttcctttttaatatgcttaaaataagcaggtggatctatttcatgtttttgatcaaaaactatttgggatatgtatgggtagggtaaatcagtaagaggtgttatttggaaccttgttttggacagtttaccagttgccttttatcccaaagttgttgtaacctgctgtgatacgatgcttcaagagaaaatgcggttataaaaaatggttcagaattaaacttttaattcattcgattg

SEQ ID NO: 9 - RNA, 159 nt, Homo sapiens; identical to SEQ ID NO: 4
  source 1..159: mol_type = mRNA

SEQ ID NO: 10 - RNA, 290 nt, Homo sapiens
  source 1..290: mol_type = mRNA
gagtaacaatacaaatggattttgggagtgactcaagaagtgaagaatgcacaagaatggatcacaagatggaatttatcaaaccctagccttgcttgttaaatttttttttttttttttttaagaatatctgtaatggtactgactttgcttgctttgaagtagctctttttttttttttttttttttttttgcagtaactgttttttaagtctctcgtagtgttaagttatagtgaatactgctacagcaatttctaatttttaagaattgagtaatggtgtagaaca

SEQ ID NO: 11 - RNA, 296 nt, Homo sapiens
  source 1..296: mol_type = mRNA
gtaactgttttttaagtctctcgtagtgttaagttatagtgaatactgctacagcaatttctaatttttaagaattgagtaatggtgtagaacactaattcataatcactctaattaattgtaatctgaataaagtgtaacaattgtgtagcctttttgtataaaatagacaaatagaaaatggtccaattagtttcctttttaatatgcttaaaataagcaggtggatctatttcatgtttttgatcaaaaactatttgggatatgtatgggtagggtaaatcagtaagaggtgt

SEQ ID NO: 12 - RNA, 248 nt, Homo sapiens
  source 1..248: mol_type = mRNA
tggtccaattagtttcctttttaatatgcttaaaataagcaggtggatctatttcatgtttttgatcaaaaactatttgggatatgtatgggtagggtaaatcagtaagaggtgttatttggaaccttgttttggacagtttaccagttgccttttatcccaaagttgttgtaacctgctgtgatacgatgcttcaagagaaaatgcggttataaaaaatggttcagaattaaacttttaattcattc

SEQ ID NO: 13 - RNA, 455 nt, Homo sapiens
  source 1..455: mol_type = mRNA
ctgtattgtctgaacttgcattgtgattggcctgtagagttgctgagagggctcgaggggtgggctggtatctcagaaagtgcctgacacactaaccaagctgagtttcctatgggaacaattgaagtaaactttttgttctggtcctttttggtcgaggtaactgttttttaagtctctcgtagtgttaagttatagtgaatactgctacagcaatttctaatttttaagaattgagtaatggtgtagaacactaattcataatcactctaattaattgtaatctgaataaagtgtaacaattgtgtagcctttttgtataaaatagacaaatagaaaatggtccaattagtttcctttttaatatgcttaaaataagcaggtggatctatttcatgtttttgatcaaaaactatttgggatatgtatgggtagggtaaatcagtaagaggtgt

SEQ ID NO: 14 - RNA, 492 nt, Homo sapiens
  source 1..492: mol_type = mRNA
gagtaacaatacaaatggattttgggagtgactcaagaagtgaagaatgcacaagaatggatcacaagatggaatttatcaaaccctagccttgcttgttaaatttttttttttttttttttaagaatatctgtaatggtactgactttgcttgctttgaagtagctctttttttttttttttttttttttttgcagtaactgttttttaagtctctcgtagtgttaagttatagtgaatactgctacagcaatttctaatttttaagaattgagtaatggtgtagaacactaattcataatcactctaattaattgtaatctgaataaagtgtaacaattgtgtagcctttttgtataaaatagacaaatagaaaatggtccaattagtttcctttttaatatgcttaaaataagcaggtggatctatttcatgtttttgatcaaaaactatttgggatatgtatgggtagggtaaatcagtaagaggtgt

SEQ ID NO: 15 - RNA, 429 nt, Homo sapiens
  source 1..429: mol_type = mRNA
gtaactgttttttaagtctctcgtagtgttaagttatagtgaatactgctacagcaatttctaatttttaagaattgagtaatggtgtagaacactaattcataatcactctaattaattgtaatctgaataaagtgtaacaattgtgtagcctttttgtataaaatagacaaatagaaaatggtccaattagtttcctttttaatatgcttaaaataagcaggtggatctatttcatgtttttgatcaaaaactatttgggatatgtatgggtagggtaaatcagtaagaggtgttatttggaaccttgttttggacagtttaccagttgccttttatcccaaagttgttgtaacctgctgtgatacgatgcttcaagagaaaatgcggttataaaaaatggttcagaattaaacttttaattcattc

SEQ ID NO: 16 - DNA, 26 bp, synthetic construct
  source 1..26: mol_type = other DNA
tgttactcctaaaggatgatttacag

SEQ ID NO: 17 - DNA, 28 bp, synthetic construct
  source 1..28: mol_type = other DNA
agacaatacagctaaaggatgatttaca

SEQ ID NO: 18 - DNA, 23 bp, synthetic construct
  source 1..23: mol_type = other DNA
taaaccactcccaccctaccaac

SEQ ID NO: 19 - DNA, 31 bp, synthetic construct
  source 1..31: mol_type = other DNA
aaaaggatccatggctactcaagctgatttg

SEQ ID NO: 20 - DNA, 31 bp, synthetic construct
  source 1..31: mol_type = other DNA
aaaatctagattacaggtcagtatcaaacca

SEQ ID NO: 21 - DNA, 27 bp, synthetic construct
  source 1..27: mol_type = other DNA
gggatccaggatacagcggcttctgcg

SEQ ID NO: 22 - DNA, 33 bp, synthetic construct
  source 1..33: mol_type = other DNA
atgagatcttgtccacgctggattttcaaaaca

SEQ ID NO: 23 - DNA, 32 bp, synthetic construct
  source 1..32: mol_type = other DNA
gctctagaatcatcctttaggagtaacaatac

SEQ ID NO: 24 - DNA, 31 bp, synthetic construct
  source 1..31: mol_type = other DNA
gctctagaatcatcctttagctgtattgtct

SEQ ID NO: 25 - DNA, 32 bp, synthetic construct
  source 1..32: mol_type = other DNA
gctctagaatcatcctttaggtaagaagttta

SEQ ID NO: 26 - DNA, 30 bp, synthetic construct
  source 1..30: mol_type = other DNA
atgggccccaatcgaatgaattaaaagttt

SEQ ID NO: 27 - DNA, 27 bp, synthetic construct
  source 1..27: mol_type = other DNA
ccggatccaggatacagcggcttctgc

SEQ ID NO: 28 - DNA, 38 bp, synthetic construct
  source 1..38: mol_type = other DNA
cagggtcgaccaatcgaatgaattaaaagtttaattct

SEQ ID NO: 29 - DNA, 27 bp, synthetic construct
  source 1..27: mol_type = other DNA
ggaagcttaggatacagcggcttctgc

SEQ ID NO: 30 - DNA, 27 bp, synthetic construct
  source 1..27: mol_type = other DNA
ggccatggtgtccacgctggattttca

SEQ ID NO: 31 - DNA, 30 bp, synthetic construct
  source 1..30: mol_type = other DNA
attctagagatactgacctgtaaatcatcc

SEQ ID NO: 32 - DNA, 35 bp, synthetic construct
  source 1..35: mol_type = other DNA
catctagaaatgaattaaaagtttaattctgaacc

SEQ ID NO: 33 - DNA, 37 bp, synthetic construct
  source 1..37: mol_type = other DNA
gccgtgtaattctagaatcatcctttaggagtaacaa

SEQ ID NO: 34 - DNA, 37 bp, synthetic construct
  source 1..37: mol_type = other DNA
gccgtgtaattctagaatcatcctttagctgtattgt

SEQ ID NO: 35 - DNA, 37 bp, synthetic construct
  source 1..37: mol_type = other DNA
gccgtgtaattctagaatcatcctttaggtaagaagt

SEQ ID NO: 36 - DNA, 36 bp, synthetic construct
  source 1..36: mol_type = other DNA
ccgccccgactctagacaatcgaatgaattaaaagt

SEQ ID NO: 37 - RNA, 600 nt, Homo sapiens
  source 1..600: mol_type = mRNA
gcggactatgacttagttgcgttacaccctttcttgacaaaacctaacttgcgcagaaaacaagatgagattggcatggctttatttgttttttttgttttgttttggttttttttttttttttggcttgactcaggatttaaaaactggaacggtgaaggtgacagcagtcggttggagcgagcatcccccaaagttcacaatgtggccgaggactttgattgcacattgttgtttttttaatagtcattccaaatatgagatgcgttgttacaggaagtcccttgccatcctaaaagccaccccacttctctctaaggagaatggcccagtcctctcccaagtccacacaggggaggtgatagcattgctttcgtgtaaattatgtaatgcaaaatttttttaatcttcgccttaatacttttttattttgttttattttgaatgatgagccttcgtgcccccccttcccccttttttgtcccccaacttgagatgtatgaaggcttttggtctccctgggagtgggtggaggcagccagggcttacctgtacactgacttgagaccagttgaataaaagtgcacaccttaaaaatga

SEQ ID NO: 38 - DNA, 24 bp, synthetic construct
  source 1..24: mol_type = other DNA
gccgcgacgcgttcgatagatcca

SEQ ID NO: 39 - DNA, 24 bp, synthetic construct
  source 1..24: mol_type = other DNA
tggatctatcgaacgcgtcgcggc

SEQ ID NO: 40 - DNA, 24 bp, synthetic construct
  source 1..24: mol_type = other DNA
gacgcgtatggtgagcaagggcga

SEQ ID NO: 41 - DNA, 29 bp, synthetic construct
  source 1..29: mol_type = other DNA
tctagattaagctcgagatctgagtccgg

SEQ ID NO: 42 - DNA, 34 bp, synthetic construct
  source 1..34: mol_type = other DNA
ccctctagataggcggactatgacttagttgcgt

SEQ ID NO: 43 - DNA, 33 bp, synthetic construct
  source 1..33: mol_type = other DNA
gcggggccctcatttttaaggtgtgcactttta

SEQ ID NO: 44 - DNA, 268 bp, synthetic construct
  source 1..268: mol_type = other DNA
aggatacagcggcttctgcgcgacttataagagctccttgtgcggcgccattttaagcctctcggtctgtggcagcagcgttggcccggccccgggagcggagagcgaggggaggcggagacggaggaaggtctgaggagcagcttcagtccccgccgagccgccaccgcaggtcgaggacggtcggactcccgcggcgggaggagcctgttcccctgagggtatttgaagtataccatacaactgttttgaaaatccagcgtggaca

SEQ ID NO: 45 - DNA, 31 bp, synthetic construct
  source 1..31: mol_type = other DNA
ccctctagactgtattgtctgaacttgcatt

SEQ ID NO: 46 - DNA, 34 bp, synthetic construct
  source 1..34: mol_type = other DNA
cccgtcgacgagagacttaaaaaacagttactgc

SEQ ID NO: 47 - DNA, 33 bp, synthetic construct
  source 1..33: mol_type = other DNA
ccctctagagagtaacaatacaaatggattttg

SEQ ID NO: 48 - DNA, 33 bp, synthetic construct
  source 1..33: mol_type = other DNA
cccgtcgactgttctacaccattactcaattct

SEQ ID NO: 49 - DNA, 33 bp, synthetic construct
  source 1..33: mol_type = other DNA
ccctctagagtaactgttttttaagtctctcgt

SEQ ID NO: 50 - DNA, 32 bp, synthetic construct
  source 1..32: mol_type = other DNA
cccgtcgacacacctcttactgatttacccta

SEQ ID NO: 51 - DNA, 33 bp, synthetic construct
  source 1..33: mol_type = other DNA
ccctctagatggtccaattagtttcctttttaa

SEQ ID NO: 52 - DNA, 32 bp, synthetic construct
  source 1..32: mol_type = other DNA
cccgtcgaccaatcgaatgaattaaaagttta

SEQ ID NO: 53 - DNA, 33 bp, synthetic construct
  source 1..33: mol_type = other DNA
ccctctagatctagagatactgacctgtaaatc

SEQ ID NO: 54 - DNA, 31 bp, synthetic construct
  source 1..31: mol_type = other DNA
cccgtcgacctgtataaagagagaaaggctg

SEQ ID NO: 55 - DNA, 28 bp, synthetic construct
  source 1..28: mol_type = other DNA
ggtctagaatacctgtccgcctttctcc

SEQ ID NO: 56 - DNA, 27 bp, synthetic construct
  source 1..27: mol_type = other DNA
ccgtcgaccgctctgctaatcctgtta

SEQ ID NO: 57 - DNA, 31 bp, synthetic construct
  source 1..31: mol_type = other DNA
atatctagactgtattgtctgaacttgcatt

SEQ ID NO: 58 - DNA, 34 bp, synthetic construct
  source 1..34: mol_type = other DNA
atagggcccgagagacttaaaaaacagttactgc

SEQ ID NO: 59 - DNA, 33 bp, synthetic construct; identical to SEQ ID NO: 49
  source 1..33: mol_type = other DNA

SEQ ID NO: 60 - DNA, 32 bp, synthetic construct
  source 1..32: mol_type = other DNA
cgcgggccctagggtaaatcagtaagaggtgt

SEQ ID NO: 61 - DNA, 33 bp, synthetic construct
  source 1..33: mol_type = other DNA
atagggcccgtaactgttttttaagtctctcgt

SEQ ID NO: 62 - DNA, 32 bp, synthetic construct
  source 1..32: mol_type = other DNA
ataggtacctagggtaaatcagtaagaggtgt

SEQ ID NO: 63 - RNA, 32 nt, synthetic construct
  source 1..32: mol_type = other RNA
gtcctttttggtcgaggtaactgttttttaag

SEQ ID NO: 64 - DNA, 32 bp, synthetic construct
  source 1..32: mol_type = other DNA
cttaaaaaacagttacctcgaccaaaaaggac

SEQ ID NO: 65 - DNA, 33 bp, synthetic construct
  source 1..33: mol_type = other DNA
cccgtcgacttacttgtacagctcgtccatgcc

SEQ ID NO: 66 - DNA, 27 bp, synthetic construct
  source 1..27: mol_type = other DNA
cccggatccatggtgagcaagggcgag

SEQ ID NO: 67 - DNA, 29 bp, synthetic construct
  source 1..29: mol_type = other DNA
cccgaattcaggatacagcggcttctgcg

SEQ ID NO: 68 - DNA, 29 bp, synthetic construct
  source 1..29: mol_type = other DNA
cccgtcgactgtccacgctggattttcaa

SEQ ID NO: 69 - DNA, 33 bp, synthetic construct
  source 1..33: mol_type = other DNA
cccggatccgagtaacaatacaaatggattttg

SEQ ID NO: 70 - DNA, 32 bp, synthetic construct
  source 1..32: mol_type = other DNA
cgcgggccccaatcgaatgaattaaaagttta

SEQ ID NO: 71 - DNA, 33 bp, synthetic construct
  source 1..33: mol_type = other DNA
cccggatccgtaactgttttttaagtctctcgt

SEQ ID NO: 72 - DNA, 30 bp, synthetic construct
  source 1..30: mol_type = other DNA
cgcgggcccacacctcttactgatttaccc

SEQ ID NO: 73 - DNA, 20 bp, synthetic construct
  source 1..20: mol_type = other DNA
taatacgactcactataggg

SEQ ID NO: 74 - DNA, 43 bp, synthetic construct
  source 1..43: mol_type = other DNA
aaataatacgactcactatagggaggatacagcggcttctgcg

SEQ ID NO: 75 - DNA, 19 bp, synthetic construct
  source 1..19: mol_type = other DNA
cggaaagatcgccgtgtaa

SEQ ID NO: 76 - DNA, 25 bp, synthetic construct
  source 1..25: mol_type = other DNA
gagagacttaaaaaacagttactgc

SEQ ID NO: 77 - DNA, 23 bp, synthetic construct
  source 1..23: mol_type = other DNA
acacctcttactgatttacccta